European Patent Application EP 4 450 519 A1, published October 23, 2024. Title: Polypeptides that binds to proangiogenic growth factors. Applicant: CENTRO DE INGENIERIA GENETICA Y BIOTECNOLOGIA. Application CU 2021 0101, filed December 15, 2021. The sequence listing filed with the application follows.

SEQUENCE LISTING (38 sequences)

SEQ ID NO: 1 - DNA, 84 bp, synthetic construct
  misc_feature 1..84: note = CDR3 Diversification, mutagenic oligonucleotide
  source 1..84: mol_type = other DNA
ggtgccttggccccaknnknnknnknnknnknnknnknnknnknnknnknnknnknnknnknnknnknngcaataatacaccgc

SEQ ID NO: 2 - DNA, 39 bp, synthetic construct
  misc_feature 1..39: note = cloning into pHG1m phagemid vector (direction 5)
  source 1..39: mol_type = other DNA
tctcacagtgcacaggtgcagctggtggaaagcggaggg

SEQ ID NO: 3 - DNA, 40 bp, synthetic construct
  misc_feature 1..40: note = cloning into pHG1m phagemid vector (direction 3)
  source 1..40: mol_type = other DNA
tatttaaagcggccgcgctgctcacggtcactaaggtgcc

SEQ ID NO: 4 - DNA, 453 bp, synthetic construct
  misc_feature 1..453: note = Nb7 DNA Sequence
  source 1..453: mol_type = other DNA
caggtgcagctggtggaaagcggagggggccttgtgcagccgggtggcagcttgcgtcttagctgcgctgcgagcggcggtagcgaatacagctattccaccttcagcctgggctggtttcgtcaggcaccgggccagggcctggaagcggtggcggcgattgcgagcatgggtgggctgacctattatgcggatagcgtgaaaggccgtttcaccattagccgggataactccaagaacacgctgtacctgcagatgaatagcctgcgtgcggaagatacggcggtgtattattgcgaaattacttcccatgcgtcgcataatgatgcgtggagtacgccgaggacggtgtggggccaaggcaccttagtgaccgtgagcagcgcggccgctggatccgaacaaaagctgatctcagaagaagacctaaactcacatcaccatcaccatcac

SEQ ID NO: 5 - DNA, 453 bp, synthetic construct
  misc_feature 1..453: note = Nb-A5 DNA sequence
  source 1..453: mol_type = other DNA
caggtgcagctggtggaaagcggagggggccttgtgcagccgggtggcagcttgcgtcttagctgcgctgcgagcggcggtagcgaatacagctattccaccttcagcctgggctggtttcgtcaggcaccgggccagggcctggaagcggtggcggcgattgcgagcatgggtgggctgacctattatgcggatagcgtgaaaggccgtttcaccattagccgggataactccaagaacacgctgtacctgcagatgaatagcctgcgtgcggaagatacggcggtgtattattgcacggctctgtatgagcgtcagccgcagctggcggcgacgaaggtggcgcggaagtggggccaaggcaccttagtgaccgtgagcagcgcggccgctggatccgaacaaaagctgatctcagaagaagacctaaactcacatcaccatcaccatcac

SEQ ID NO: 6 - DNA, 53 bp, synthetic construct
  misc_feature 1..53: note = Oligonucleotide to extract from phagemid for pACR
  source 1..53: mol_type = other DNA
attctcccatggcgtctcacagtgcacaggtgcagctggtggaaagcggaggg

SEQ ID NO: 7 - DNA, 54 bp, synthetic construct
  misc_feature 1..54: note = Oligonucleotide to extract from phagemid for pACR
  source 1..54: mol_type = other DNA
aaggaaaatcgccggcgtatttaaagcggccgtgctcacggtcactaaggtgcc

SEQ ID NO: 8 - DNA, 89 bp, synthetic construct
  misc_feature 1..89: note = CDR1 Diversification, mutagenic oligonucleotide (direction 3)
  source 1..89: mol_type = other DNA
cttccaggccctggcccggtgcctgacgaaaccamnnmnnmnnmnnmnnmnnmnnmnnmnnmnnmnnmngccgctcgcagcgcagctaa

SEQ ID NO: 9 - DNA, 92 bp, synthetic construct
  misc_feature 1..92: note = CDR2 Diversification, mutagenic oligonucleotide (direction 5)
  source 1..92: mol_type = other DNA
tcaggcaccgggccagggcctggaagcggtggcggcgattnnknnknnknnknnknngggnnkacctattatgcggatagcgtgaaaggccg

SEQ ID NO: 10 - DNA, 459 bp, synthetic construct
  misc_feature 1..459: note = Nb-V1 DNA sequence
  source 1..459: mol_type = other DNA
caggtgcagctggtggaaagcggagggggccttgtgcagccgggtggcagcttgcgtcttagctgcgctgcgagcggcaattctgcggaagataggctgtataattcttatacttggtttcgtcaggcaccgggccagggcctggaagcggtggcggcgattagtagtcatttttctgcggggttgacctattatgcggatagcgtgaaaggccgtttcaccattagccgggataactccaagaacacgctgtacctgcagatgaatagcctgcgtgcggaagatacggcggtgtattattgcgaaattacttcccatgcgtcgcataatgatgcgtggagtacgccgaggacggtgtggggccaaggcaccttagtgaccgtgagcagcgcggccgctggatccgaacaaaagctgatctcagaagaagacctaaactcacatcaccatcaccatcac

SEQ ID NO: 11 - DNA, 459 bp, synthetic construct
  misc_feature 1..459: note = Nb-F3 DNA sequence
  source 1..459: mol_type = other DNA
caggtgcagctggtggaaagcggagggggccttgtgcagccgggtggcagcttgcgtcttagctgcgctgcgagcggcactcaggatgggcggctgcttacgctggggggttcttggtttcgtcaggcaccgggccagggcctggaagcggtggcggcgattggggcgggggatagggggggggcgacctattatgcggatagcgtgaaaggccgtttcaccattagccgggataactccaagaacacgctgtacctgcagatgaatagcctgcgtgcggaagatacggcggtgtattattgcacggctctgtatgagcgtcagccgcagctggcggcgacgaaggtggcgcggaagtggggccaaggcaccttagtgaccgtgagcagcgcggccgctggatccgaacaaaagctgatctcagaagaagacctaaactcacatcaccatcaccatcac

SEQ ID NO: 12 - protein, 153 aa, synthetic construct
  REGION 1..153: note = Nb-V1 sequence
QVQLVESGGGLVQPGGSLRLSCAASGNSAEDRLYNSYTWFRQAPGQGLEAVAAISSHFSAGLTYYADSVKGRFTISRDNSKNTLYLQMNSLRAEDTAVYYCEITSHASHNDAWSTPRTVWGQGTLVTVSSAAAGSEQKLISEEDLNSHHHHHH

SEQ ID NO: 13 - protein, 153 aa, synthetic construct
  REGION 1..153: note = Nb-F3 Sequence
QVQLVESGGGLVQPGGSLRLSCAASGTEDGRLLTLGGSWFRQAPGQGLEAVAAIGAGDRGGATYYADSVKGRFTISRDNSKNTLYLQMNSLRAEDTAVYYCTALYERQPQLAATKVARKWGQGTLVTVSSAAAGSEQKLISEEDLNSHHHHHH

SEQ ID NO: 14 - DNA, 22 bp, synthetic construct
  misc_feature 1..22: note = oligonucleotide for cloning into pACR1k (direction 5)
  source 1..22: mol_type = other DNA
ttgctgctgctggcagctcagc

SEQ ID NO: 15 - DNA, 45 bp, synthetic construct
  misc_feature 1..45: note = Oligonucleotide for bispecific and bivalent constructions (direction 3)
  source 1..45: mol_type = other DNA
tttggagctggggtcttcgctgtggtgcgcgctgctcacggtcac

SEQ ID NO: 16 - DNA, 45 bp, synthetic construct
  misc_feature 1..45: note = Oligonucleotide for bispecific and bivalent constructions (direction 5')
  source 1..45: mol_type = other DNA
gaccccagctccaaagctcccaaagctcccgcacaggtgcagctg

SEQ ID NO: 17 - DNA, 20 bp, synthetic construct
  misc_feature 1..20: note = Oligonucleotide for cloning into pACR1k (direction 3')
  source 1..20: mol_type = other DNA
tttgttcggatccagcggcc

SEQ ID NO: 18 - protein, 299 aa, synthetic construct
  REGION 1..299: note = Nb-VF3 sequence
QVQLVESGGGLVQPGGSLRLSCAASGNSAEDRLYNSYTWFRQAPGQGLEAVAAISSHFSAGLTYYADSVKGRFTISRDNSKNTLYLQMNSLRAEDTAVYYCEITSHASHNDAWSTPRTVWGQGTLVTVSSAHHSEDPSSKAPKAPAQVQLVESGGGLVQPGGSLRLSCAASGTEDGRLLTLGGSWFRQAPGQGLEAVAAIGAGDRGGATYYADSVKGRFTISRDNSKNTLYLQMNSLRAEDTAVYYCTALYERQPQLAATKVARKWGQGTLVTVSSAAAGSEQKLISEEDLNSHHHHHH

SEQ ID NO: 19 - protein, 299 aa, synthetic construct
  REGION 1..299: note = Nb-FV1 sequence
QVQLVESGGGLVQPGGSLRLSCAASGTEDGRLLTLGGSWFRQAPGQGLEAVAAIGAGDRGGATYYADSVKGRFTISRDNSKNTLYLQMNSLRAEDTAVYYCTALYERQPQLAATKVARKWGQGTLVTVSSAHHSEDPSSKAPKAPAQVQLVESGGGLVQPGGSLRLSCAASGNSAEDRLYNSYTWFRQAPGQGLEAVAAISSHFSAGLTYYADSVKGRFTISRDNSKNTLYLQMNSLRAEDTAVYYCEITSHASHNDAWSTPRTVWGQGTLVTVSSAAAGSEQKLISEEDLNSHHHHHH

SEQ ID NO: 20 - protein, 299 aa, synthetic construct
  REGION 1..299: note = Nb-VV6 Sequence
QVQLVESGGGLVQPGGSLRLSCAASGNSAEDRLYNSYTWFRQAPGQGLEAVAAISSHFSAGLTYYADSVKGRFTISRDNSKNTLYLQMNSLRAEDTAVYYCEITSHASHNDAWSTPRTVWGQGTLVTVSSAHHSEDPSSKAPKAPAQVQLVESGGGLVQPGGSLRLSCAASGNSAQDRLYNSYTWFRQAPGQGLEAVAAISSHFSAGLTYYADSVKGRFTISRDNSKNTLYLQMNSLRAEDTAVYYCEITSHASHNDAWSTPRTVWGQGTLVTVSSAAAGSEQKLISEEDLNSHHHHHH

SEQ ID NO: 21 - protein, 299 aa, synthetic construct
  REGION 1..299: note = Nb-FF2 Sequence
QVQLVESGGGLVQPGGSLRLSCAASGTEDGRLLTLGGSWFRQAPGQGLEAVAAIGAGDRGGATYYADSVKGRFTISRDNSKNTLYLQMNSLRAEDTAVYYCTALYERQPQLAATKVARKWGQGTLVTVSSAHHSEDPSSKAPKAPAQVQLVESGGGLVQPGGSLRLSCAASGTEDGRLLTLGGSWFRQAPGQGLEAVAAIGAGDRGGATYYADSVKGRFTISRDNSKNTLYLQMNSLRAEDTAVYYCTALYERQPQLAATKVARKWGQGTLVTVSSAAAGSEQKLISEEDLNSHHHHHH

SEQ ID NO: 22 - DNA, 33 bp, synthetic construct
  misc_feature 1..33: note = Oligonucleotide for removal of c-myc fragments and histidine tag
  source 1..33: mol_type = other DNA
acacacagatctttattattagctctcacgggt

SEQ ID NO: 23 - protein, 130 aa, synthetic construct
  REGION 1..130: note = Nb-V1 sequence without cmyc or H6
QVQLVESGGGLVQPGGSLRLSCAASGNSAEDRLYNSYTWFRQAPGQGLEAVAAISSHFSAGLTYYADSVKGRFTISRDNSKNTLYLQMNSLRAEDTAVYYCEITSHASHNDAWSTPRTVWGQGTLVTVSS

SEQ ID NO: 24 - protein, 130 aa, synthetic construct
  REGION 1..130: note = Nb-F3 sequence without cmyc or H6
QVQLVESGGGLVQPGGSLRLSCAASGTEDGRLLTLGGSWFRQAPGQGLEAVAAIGAGDRGGATYYADSVKGRFTISRDNSKNTLYLQMNSLRAEDTAVYYCTALYERQPQLAATKVARKWGQGTLVTVSS

SEQ ID NO: 25 - protein, 276 aa, synthetic construct
  REGION 1..276: note = Nb-VV6 sequence without cmyc or H6
QVQLVESGGGLVQPGGSLRLSCAASGNSAEDRLYNSYTWFRQAPGQGLEAVAAISSHFSAGLTYYADSVKGRFTISRDNSKNTLYLQMNSLRAEDTAVYYCEITSHASHNDAWSTPRTVWGQGTLVTVSSAHHSEDPSSKAPKAPAQVQLVESGGGLVQPGGSLRLSCAASGNSAQDRLYNSYTWFRQAPGQGLEAVAAISSHFSAGLTYYADSVKGRFTISRDNSKNTLYLQMNSLRAEDTAVYYCEITSHASHNDAWSTPRTVWGQGTLVTVSS

SEQ ID NO: 26 - protein, 276 aa, synthetic construct
  REGION 1..276: note = Nb-FF2 sequence without cmyc or H6
QVQLVESGGGLVQPGGSLRLSCAASGTEDGRLLTLGGSWFRQAPGQGLEAVAAIGAGDRGGATYYADSVKGRFTISRDNSKNTLYLQMNSLRAEDTAVYYCTALYERQPQLAATKVARKWGQGTLVTVSSAHHSEDPSSKAPKAPAQVQLVESGGGLVQPGGSLRLSCAASGTEDGRLLTLGGSWFRQAPGQGLEAVAAIGAGDRGGATYYADSVKGRFTISRDNSKNTLYLQMNSLRAEDTAVYYCTALYERQPQLAATKVARKWGQGTLVTVSS

SEQ ID NO: 27 - protein, 276 aa, synthetic construct
  REGION 1..276: note = Nb-FV1 sequence without cmyc or H6
QVQLVESGGGLVQPGGSLRLSCAASGTEDGRLLTLGGSWFRQAPGQGLEAVAAIGAGDRGGATYYADSVKGRFTISRDNSKNTLYLQMNSLRAEDTAVYYCTALYERQPQLAATKVARKWGQGTLVTVSSAHHSEDPSSKAPKAPAQVQLVESGGGLVQPGGSLRLSCAASGNSAEDRLYNSYTWFRQAPGQGLEAVAAISSHFSAGLTYYADSVKGRFTISRDNSKNTLYLQMNSLRAEDTAVYYCEITSHASHNDAWSTPRTVWGQGTLVTVSS

SEQ ID NO: 28 - protein, 276 aa, synthetic construct
  REGION 1..276: note = Nb-VF3 sequence without cmyc or H6
QVQLVESGGGLVQPGGSLRLSCAASGNSAEDRLYNSYTWFRQAPGQGLEAVAAISSHFSAGLTYYADSVKGRFTISRDNSKNTLYLQMNSLRAEDTAVYYCEITSHASHNDAWSTPRTVWGQGTLVTVSSAHHSEDPSSKAPKAPAQVQLVESGGGLVQPGGSLRLSCAASGTEDGRLLTLGGSWFRQAPGQGLEAVAAIGAGDRGGATYYADSVKGRFTISRDNSKNTLYLQMNSLRAEDTAVYYCTALYERQPQLAATKVARKWGQGTLVTVSS

SEQ ID NO: 29 - DNA, 18 bp, synthetic construct
  misc_feature 1..18: note = Oligonucleotide for cloning into pVSJG-huFc (direction 5)
  source 1..18: mol_type = other DNA
gcttaagcaggtgcagct

SEQ ID NO: 30 - DNA, 23 bp, synthetic construct
  misc_feature 1..23: note = Oligonucleotide for cloning into pVSJG-huFc (direction 3)
  source 1..23: mol_type = other DNA
tctagagctgctcacggtcacta

SEQ ID NO: 31 - protein, 374 aa, synthetic construct
  REGION 1..374: note = Nb-V1-hFc sequence
QVQLVESGGGLVQPGGSLRLSCAASGNSAEDRLYNSYTWFRQAPGQGLEAVAAISSHFSAGLTYYADSVKGRFTISRDNSKNTLYLQMNSLRAEDTAVYYCEITSHASHNDAWSTPRTVWGQGTLVTVSSRGGGGSGGGGSAEPKSCDKTHTCPPCPAPELLGGPSVFLFPPKPKDTLMISRTPEVTCVVVDVSHEDPEVKFNWYVDGVKVHNAKTKPREEQYNSTYRVVSVLTVLHQDWLNGKEYKCKVSNKALPAPIEKTISKAKGQPREPQVYTLPPSREEMTKNQVSLTCLVKGFYPSDIAVEWESNGQPENNYKTTPPVLDSDGSFFLYSKLTVDKSRWQQGNVFSCSVMHEALHNHYTQKSLSLSPGK

SEQ ID NO: 32 - protein, 374 aa, synthetic construct
  REGION 1..374: note = Nb-F3-hFc sequence
QVQLVESGGGLVQPGGSLRLSCAASGTEDGRLLTLGGSWFRQAPGQGLEAVAAIGAGDRGGATYYADSVKGRFTISRDNSKNTLYLQMNSLRAEDTAVYYCTALYERQPQLAATKVARKWGQGTLVTVSSRGGGGSGGGGSAEPKSCDKTHTCPPCPAPELLGGPSVFLFPPKPKDTLMISRTPEVTCVVVDVSHEDPEVKFNWYVDGVKVHNAKTKPREEQYNSTYRVVSVLTVLHQDWLNGKEYKCKVSNKALPAPIEKTISKAKGQPREPQVYTLPPSREEMTKNQVSLTCLVKGFYPSDIAVEWESNGQPENNYKTTPPVLDSDGSFFLYSKLTVDKSRWQQGNVFSCSVMHEALHNHYTQKSLSLSPGK

SEQ ID NO: 33 - protein, 520 aa, synthetic construct
  REGION 1..520: note = Nb-VV6-hFc sequence
QVQLVESGGGLVQPGGSLRLSCAASGNSAEDRLYNSYTWFRQAPGQGLEAVAAISSHFSAGLTYYADSVKGRFTISRDNSKNTLYLQMNSLRAEDTAVYYCEITSHASHNDAWSTPRTVWGQGTLVTVSSAHHSEDPSSKAPKAPAQVQLVESGGGLVQPGGSLRLSCAASGNSAQDRLYNSYTWFRQAPGQGLEAVAAISSHFSAGLTYYADSVKGRFTISRDNSKNTLYLQMNSLRAEDTAVYYCEITSHASHNDAWSTPRTVWGQGTLVTVSSRGGGGSGGGGSAEPKSCDKTHTCPPCPAPELLGGPSVFLFPPKPKDTLMISRTPEVTCVVVDVSHEDPEVKFNWYVDGVKVHNAKTKPREEQYNSTYRVVSVLTVLHQDWLNGKEYKCKVSNKALPAPIEKTISKAKGQPREPQVYTLPPSREEMTKNQVSLTCLVKGFYPSDIAVEWESNGQPENNYKTTPPVLDSDGSFFLYSKLTVDKSRWQQGNVFSCSVMHEALHNHYTQKSLSLSPGK

SEQ ID NO: 34 - protein, 520 aa, synthetic construct
  REGION 1..520: note = Nb-FF2-hFc sequence
QVQLVESGGGLVQPGGSLRLSCAASGTEDGRLLTLGGSWFRQAPGQGLEAVAAIGAGDRGGATYYADSVKGRFTISRDNSKNTLYLQMNSLRAEDTAVYYCTALYERQPQLAATKVARKWGQGTLVTVSSAHHSEDPSSKAPKAPAQVQLVESGGGLVQPGGSLRLSCAASGTEDGRLLTLGGSWFRQAPGQGLEAVAAIGAGDRGGATYYADSVKGRFTISRDNSKNTLYLQMNSLRAEDTAVYYCTALYERQPQLAATKVARKWGQGTLVTVSSRGGGGSGGGGSAEPKSCDKTHTCPPCPAPELLGGPSVFLFPPKPKDTLMISRTPEVTCVVVDVSHEDPEVKFNWYVDGVKVHNAKTKPREEQYNSTYRVVSVLTVLHQDWLNGKEYKCKVSNKALPAPIEKTISKAKGQPREPQVYTLPPSREEMTKNQVSLTCLVKGFYPSDIAVEWESNGQPENNYKTTPPVLDSDGSFFLYSKLTVDKSRWQQGNVFSCSVMHEALHNHYTQKSLSLSPGK

SEQ ID NO: 35 - protein, 520 aa, synthetic construct
  REGION 1..520: note = Nb-FV1-hFc Sequence
QVQLVESGGGLVQPGGSLRLSCAASGTEDGRLLTLGGSWFRQAPGQGLEAVAAIGAGDRGGATYYADSVKGRFTISRDNSKNTLYLQMNSLRAEDTAVYYCTALYERQPQLAATKVARKWGQGTLVTVSSAHHSEDPSSKAPKAPAQVQLVESGGGLVQPGGSLRLSCAASGNSAEDRLYNSYTWFRQAPGQGLEAVAAISSHFSAGLTYYADSVKGRFTISRDNSKNTLYLQMNSLRAEDTAVYYCEITSHASHNDAWSTPRTVWGQGTLVTVSSRGGGGSGGGGSAEPKSCDKTHTCPPCPAPELLGGPSVFLFPPKPKDTLMISRTPEVTCVVVDVSHEDPEVKFNWYVDGVKVHNAKTKPREEQYNSTYRVVSVLTVLHQDWLNGKEYKCKVSNKALPAPIEKTISKAKGQPREPQVYTLPPSREEMTKNQVSLTCLVKGFYPSDIAVEWESNGQPENNYKTTPPVLDSDGSFFLYSKLTVDKSRWQQGNVFSCSVMHEALHNHYTQKSLSLSPGK

SEQ ID NO: 36 - protein, 520 aa, synthetic construct
  REGION 1..520: note = Nb-VF3-hFc sequence
QVQLVESGGGLVQPGGSLRLSCAASGNSAEDRLYNSYTWFRQAPGQGLEAVAAISSHFSAGLTYYADSVKGRFTISRDNSKNTLYLQMNSLRAEDTAVYYCEITSHASHNDAWSTPRTVWGQGTLVTVSSAHHSEDPSSKAPKAPAQVQLVESGGGLVQPGGSLRLSCAASGTEDGRLLTLGGSWFRQAPGQGLEAVAAIGAGDRGGATYYADSVKGRFTISRDNSKNTLYLQMNSLRAEDTAVYYCTALYERQPQLAATKVARKWGQGTLVTVSSRGGGGSGGGGSAEPKSCDKTHTCPPCPAPELLGGPSVFLFPPKPKDTLMISRTPEVTCVVVDVSHEDPEVKFNWYVDGVKVHNAKTKPREEQYNSTYRVVSVLTVLHQDWLNGKEYKCKVSNKALPAPIEKTISKAKGQPREPQVYTLPPSREEMTKNQVSLTCLVKGFYPSDIAVEWESNGQPENNYKTTPPVLDSDGSFFLYSKLTVDKSRWQQGNVFSCSVMHEALHNHYTQKSLSLSPGK

SEQ ID NO: 37 - DNA, 38 bp, synthetic construct
  misc_feature 1..38: note = NotI-Kozak ret-MAQVQLV oligonucleotide
  source 1..38: mol_type = other DNA
gcggccgcaccgagaccatggctcaggtgacgctggtg

SEQ ID NO: 38 - DNA, 29 bp, synthetic construct
  misc_feature 1..29: note = PmeI-Stop-Stop-KGPSL (Fc) Oligonucleotide
  source 1..29: mol_type = other DNA
caaatttgttattatttacccggagacag